European Patent Application EP 4 360 658 A1, published May 1, 2024. Title: Compounds for Detection of Oral Inflammation. Applicant: Julius-Maximilians-Universitaet Wuerzburg. The sequence listing filed with the application follows.

SEQUENCE LISTING (42 sequences)

SEQ ID NO: 1 - protein, 8 aa, synthetic construct
  VARIANT 2: note = A or P
  VARIANT 4: note = A or E
GXLXJVGA

SEQ ID NO: 2 - protein, 8 aa, synthetic construct
GPLELVGA

SEQ ID NO: 3 - protein, 8 aa, synthetic construct
GPLEIVGA

SEQ ID NO: 4 - protein, 8 aa, synthetic construct
GPLALVGA

SEQ ID NO: 5 - protein, 8 aa, synthetic construct
GPLAIVGA

SEQ ID NO: 6 - protein, 8 aa, synthetic construct
GALELVGA

SEQ ID NO: 7 - protein, 8 aa, synthetic construct
GALEIVGA

SEQ ID NO: 8 - protein, 8 aa, synthetic construct
GALALVGA

SEQ ID NO: 9 - protein, 8 aa, synthetic construct
GALAIVGA

SEQ ID NO: 10 - protein, 8 aa, synthetic construct
GPQAYWGA

SEQ ID NO: 11 - protein, 8 aa, synthetic construct
GPLAYWGA

SEQ ID NO: 12 - protein, 8 aa, synthetic construct
GPQGIWGA

SEQ ID NO: 13 - protein, 8 aa, synthetic construct
GPQGYWGA

SEQ ID NO: 14 - protein, 8 aa, synthetic construct
GPQGIAGA

SEQ ID NO: 15 - protein, 8 aa, synthetic construct
GPQGIAGQ

SEQ ID NO: 16 - protein, 4 aa, synthetic construct
QPVV

SEQ ID NO: 17 - protein, 4 aa, synthetic construct
DAPV

SEQ ID NO: 18 - protein, 4 aa, synthetic construct
GSGS

SEQ ID NO: 19 - protein, 8 aa, synthetic construct
  SITE 1: note = acetylated glycine
  SITE 8: note = alanine comprising C-terminal functionalization with Den-CH2-NH2
GPQGIAGA

SEQ ID NO: 20 - protein, 16 aa, synthetic construct
  SITE 1: note = acetylated glycine
  SITE 16: note = serine comprising C-terminal functionalization with Den-CH2-NH2
GSGSGPQGIAGAGSGS

SEQ ID NO: 21 - protein, 8 aa, synthetic construct
  SITE 8: note = serine comprising C-terminal functionalization with Den-CH2-NH2
IAGAGSGS

SEQ ID NO: 22 - protein, 8 aa, synthetic construct
  SITE 1: note = acetylated glycine
GPQGIAGA

SEQ ID NO: 23 - protein, 16 aa, synthetic construct
  SITE 1: note = acetylated glycine
GSGSGPQGIAGAGSGS

SEQ ID NO: 24 - protein, 8 aa, synthetic construct
  SITE 1: note = acetylated glycine
GPQGIWGA

SEQ ID NO: 25 - protein, 8 aa, synthetic construct
  SITE 1: note = acetylated glycine
GPQGYWGA

SEQ ID NO: 26 - protein, 8 aa, synthetic construct
  SITE 1: note = acetylated glycine
GPQAYWGA

SEQ ID NO: 27 - protein, 8 aa, synthetic construct
  SITE 1: note = acetylated glycine
GPLAYWGA

SEQ ID NO: 28 - protein, 8 aa, synthetic construct
  SITE 1: note = acetylated glycine
GPLELVGA

SEQ ID NO: 29 - protein, 8 aa, synthetic construct
  SITE 1: note = acetylated glycine
GPLEIVGA

SEQ ID NO: 30 - protein, 8 aa, synthetic construct
  SITE 1: note = acetylated glycine
GPLALVGA

SEQ ID NO: 31 - protein, 8 aa, synthetic construct
  SITE 1: note = acetylated glycine
GPLAIVGA

SEQ ID NO: 32 - protein, 8 aa, synthetic construct
  SITE 1: note = acetylated glycine
GALELVGA

SEQ ID NO: 33 - protein, 8 aa, synthetic construct
  SITE 1: note = acetylated glycine
GALEIVGA

SEQ ID NO: 34 - protein, 8 aa, synthetic construct
  SITE 1: note = acetylated glycine
GALALVGA

SEQ ID NO: 35 - protein, 8 aa, synthetic construct
  SITE 1: note = acetylated glycine
GALAIVGA

SEQ ID NO: 36 - protein, 17 aa, synthetic construct
  SITE 1: note = acetylated glycine
  SITE 17: note = L-azidohomoalanine
GSGSGPLALVGAGSGSA

SEQ ID NO: 37 - protein, 17 aa, synthetic construct
  SITE 1: note = acetylated glycine
  SITE 17: note = L-azidohomoalanine
GSGSGALELVGAGSGSA

SEQ ID NO: 38 - protein, 17 aa, synthetic construct
  SITE 1: note = acetylated glycine
  SITE 17: note = L-azidohomoalanine
GSGSGALALVGAGSGSA

SEQ ID NO: 39 - protein, 17 aa, synthetic construct
  SITE 1: note = acetylated glycine
  SITE 17: note = L-azidohomoalanine, modified with DBCO-Sulfo-Cy5
GSGSGPLALVGAGSGSA

SEQ ID NO: 40 - protein, 17 aa, synthetic construct
  SITE 1: note = acetylated glycine
  SITE 17: note = L-azidohomoalanine, modified with AFDye488-DBCO
GSGSGALELVGAGSGSA

SEQ ID NO: 41 - protein, 17 aa, synthetic construct
  SITE 1: note = acetylated glycine
  SITE 17: note = L-azidohomoalanine, modified with Sulfo-Cy-3-Alkin
GSGSGALELVGAGSGSA

SEQ ID NO: 42 - protein, 16 aa, synthetic construct
  SITE 1: note = acetylated glycine
  SITE 16: note = serine comprising C-terminal functionalization with Den-CH2-NH2
GSGSGPQAYWGAGSGS